European Patent Application EP 4 640 834 A1, published October 29, 2025. Title: Flavanone 2-hydroxylase and use thereof. Applicant: Suntory Holdings Limited. Application JP. The sequence listing filed with the application follows.

SEQUENCE LISTING (22 sequences)

SEQ ID NO: 1 - DNA, 1083 bp, Silene vulgaris
  source 1..1083: mol_type = genomic DNA
atgacaaaagaggaatcaataaccgtgcccgaatgggaaggcgagaaatccgtgaagcaaacttacgttagggacgaagatgaccgtcctaaggtcgcttacaacgaattcagcgacgacattcccgtcatttccctctctggtatcgactcagccgacgagagggctcacattcgcagccaaatcactgaggcctgcgagaaatacggcattttccaggtcgtaaaccacggtattgacactgacctcatctctaccatggctcgtctttgttccgagttttttaatttgccgggtcatgagaagcaacgttttggtgcttctgaaggtaaacccgggagcttcttcgtctctagccccttcaagggtgagttggtaaaaaattggagagaaacggtgacgcaatgcacattcccaatcaagagcggggactacacactatggcccgacaagcccgacggatggaaagccgtgactaaggaatacagcgaaaaaatgatggacctttcccaccagctgcttgggctactatcagaggccatgggtcttgagacagaggccctaagcaaggcctgtgttacaatggaccaaagggttatgattaactactacccaaaatgccctcagccagacctcacccttggccttccccggcacaccgaccccgggaccatcacccttctctaccaggacctggttggtgggctacaagccactcgcgatgatggtaagacttggatcactgtcccgccgattgctggtgctcttgttgtcaaccttggtgatcatgcttattacgtaagtaatggaaggtttacaagtgcggaacaccgggccgtggtgaactcaaaccagagtaggttgtcaatagcaacattccaatacccaacagctgaggcaacggtcttcccattggcgataaggcaaggagagaagccggtaatggaagaagctatcaccttcgcggagatgtatagaaggaagatgagctcggacattgagcgtccgaagcttaagaagcttgatggtaaaatggacaagtccaagttagagtctaggcccatcggcgagatctttgtttga

SEQ ID NO: 2 - protein, 360 aa, Silene vulgaris
MTKEESITVPEWEGEKSVKQTYVRDEDDRPKVAYNEFSDDIPVISLSGIDSADERAHIRSQITEACEKYGIFQVVNHGIDTDLISTMARLCSEFFNLPGHEKQRFGASEGKPGSFFVSSPFKGELVKNWRETVTQCTFPIKSGDYTLWPDKPDGWKAVTKEYSEKMMDLSHQLLGLLSEAMGLETEALSKACVTMDQRVMINYYPKCPQPDLTLGLPRHTDPGTITLLYQDLVGGLQATRDDGKTWITVPPIAGALVVNLGDHAYYVSNGRFTSAEHRAVVNSNQSRLSIATFQYPTAEATVFPLAIRQGEKPVMEEAITFAEMYRRKMSSDIERPKLKKLDGKMDKSKLESRPIGEIFV

SEQ ID NO: 3 - DNA, 1083 bp, Silene vulgaris
  source 1..1083: mol_type = genomic DNA
atgacaaaagaaaaggcaacaacgttgaccgagctccaagaccaaaactgcatcaaccaaagtttcgtaagagacgaggatgaccgtcctaaggtcgcctacaacgactttaccgacgttatccccgtcatttcactctccggcattgacgcccacgatgaaagggctgaaattcgtcgtaagatcactgaagcttgcgaaacttggggccttttccaggtcatcgaccatggtgttgaacttgaaattatatcggagatggcacgcctttctaccgagttttttcacttgcccgcgtctgagaagcagcagtttgctgcttccgatggcaagccgggaagtttctttgtttcaagcccttttaagagagagttggtacagaactggagagagacagtaacacaatgcacatacccaattaagagtggggactacacattatggccagataaacctgaaggatggcgaaaaataaccaaagaatacagtgataaaatgatggagctaagtcacaaactccttgggattctttctgaggcaatgggtttagagacggacgcgttaagcaaggcttgtgtcgaaatggatcaaagggttatgatcaattattaccctaagtgccctcaacctgacctcacccttgggctccttcgccacaccgatcctggtaccattactcttctttaccaggatcangttggtgggcttcnngccacttgtgatgatggtgtgacttggnttacggttcctcctattcctggcgcgcttgttgttaaccttggtgatcattcccattttgtgagcaatggaaggttcgtgagtgcggagcacagggcagtggtgaactcgaacacaggcaggctgtcgatggtgacatttcagtatccgacagcagaggcgacagtgtaccccttgacgctgagagaaggggagacgccgatcatggaagaggccataaccttcggggagatgtacaggaggaagatgagcaaagaccttgagcttcctcggaacaagaagctagacactaagatggaaaagtcggaattagagtcaagacccattgacgccatctttatttaa

SEQ ID NO: 4 - protein, 360 aa, Silene vulgaris
MTKEKATTLTELQDQNCINQSFVRDEDDRPKVAYNDFTDVIPVISLSGIDAHDERAEIRRKITEACETWGLFQVIDHGVELEIISEMARLSTEFFHLPASEKQQFAASDGKPGSFFVSSPFKRELVQNWRETVTQCTYPIKSGDYTLWPDKPEGWRKITKEYSDKMMELSHKLLGILSEAMGLETDALSKACVEMDQRVMINYYPKCPQPDLTLGLLRHTDPGTITLLYQDXVGGLXATCDDGVTWXTVPPIPGALVVNLGDHSHFVSNGRFVSAEHRAVVNSNTGRLSMVTFQYPTAEATVYPLTLREGETPIMEEAITFGEMYRRKMSKDLELPRNKKLDTKMEKSELESRPIDAIFI

SEQ ID NO: 5 - DNA, 1092 bp, Dianthus superbus
  source 1..1092: mol_type = genomic DNA
atgacaaaagaagataaaaaaaatgttactacattgacagaattagtagaccaaaaatgcattaaccaaagcttcgtaagagacgaagacgagcgtccgaaagtcgcttacaacgaatttagcgacgaaattcccgtcatttcgctacttggcattgatgatgacagcgagaggactcacattcgtcgtaagattaccgaggcgtgtgagtcttggggtatttttcaggtcgttgaccatggagttgacctcttactcatttcggaaatggctcggcttagtaccgagttttttaacttgcccgctcatgagaagcagcggttcgatacctcgggcggtaagcccgggagttttttcgtgtcgagtccttttaagggggaactagttcagaactggcgagagacggtcacacaatgcacgtacccgatcaagagcggagacttcaacctatggccggataagccagagggttggagaaaagtaaccaaagactacggtgacaaaatgatgggcctaagtcacaagatacttgggcttttatctgaagctatgggtctcgagaccgaggcccttagcaaggcctgtgttgagatggaccaaagggttatgatcaactactaccctaagtgccctcaacccgacttaacccttggccttctccgccacactgatcctggtacaattactcttttgtaccaagatcaagttggcggtctccaagccacccgtgatgacggtgtgacttggatcactgttacgcctgttcctggtgcccttgtcgtcaatcttggtgatcatgcctattacgcgagtaacggaaggttcacaagtgcggaacaccgagcagtggtgaactcgaatcaaggcaggctgtcgatggcgacattccaatacccgacagcggaggcaatggtgtatccgttgacagtcagtgaaggcgagaagccggtgatggaagaggccatcaccttcgcggaaatgtaccgtaggaaaatgagcaaggaccttgagcgtcctcaccttaagaagctcgacaatacgatggacaagtcaaaattagagggtcgggccattaatgagatctttatctaa

SEQ ID NO: 6 - protein, 363 aa, Dianthus superbus
MTKEDKKNVTTLTELVDQKCINQSFVRDEDERPKVAYNEFSDEIPVISLLGIDDDSERTHIRRKITEACESWGIFQVVDHGVDLLLISEMARLSTEFFNLPAHEKQRFDTSGGKPGSFFVSSPFKGELVQNWRETVTQCTYPIKSGDFNLWPDKPEGWRKVTKDYGDKMMGLSHKILGLLSEAMGLETEALSKACVEMDQRVMINYYPKCPQPDLTLGLLRHTDPGTITLLYQDQVGGLQATRDDGVTWITVTPVPGALVVNLGDHAYYASNGRFTSAEHRAVVNSNQGRLSMATFQYPTAEAMVYPLTVSEGEKPVMEEAITFAEMYRRKMSKDLERPHLKKLDNTMDKSKLEGRAINEIFI

SEQ ID NO: 7 - DNA, 1086 bp, Agrostemma githago
  source 1..1086: mol_type = genomic DNA
atgcctcaagaagagtcaataataaccgtgagtgagatgcaagaggataaatccgtggagcaaaaattcgttagggacgaagatgaccgtcctaaggtcgcatacaacgaatttagcgacgacattcccgtgatttccctctccggcattgactcccccgacgacagggaccacattcgccgccaagtcacagaggcctgcgaggaatacggcattttccaagtggtagaccatggtatcgactctgatatcatctcgaccatggctcgtcaatcttcccagtttttcaacttgcccgctcctgaaaagcagcgtttcgctgctgccgagggtaaacctggcagcttcttcgtctctagtcccttcaagggtgagttggtgcaaaattggagagaaacggtgacgcagtgcacgttcccgatcaagagtggagactacacgctgtggccggacaagccggagggatggagaagcgtgaccaaggagtacagtgaaaaaatgatggatctttctcacaaactcctcggggtgctgtccgaggcaatgggtctggagacggaggccctaagcaatgcctgcgttacaatggaccaacgggttatgattaattactatcccaagtgccctcaaccggacctcaccctcggtctcccccgccacaccgaccctggcaccatcacccttctctaccaggacctcgttggtggcctccaagccactcgcgatgatggtaagacttggattactgtcccgcctattcccggtgctcttgtcgtcaaccttggcgatcatgccttttacgcaagcaacggaaggttcacaagtgcggaacaccgggcagtggtgaactcaaaccagagcaggttgtcaatagcgacattccaatatccgacagcggaggcaatggtgtaccccttagcaataagggaaggagagacagcggtgatggaagaggccatcacgtttgcggagatgtataggaggaagatgagctccgacattgagcgacctaagcataagaaggtcgatggtaaaatggacaagtccaagttagagtctaggcccatggaagagatctttgtttga

SEQ ID NO: 8 - protein, 361 aa, Agrostemma githago
MPQEESIITVSEMQEDKSVEQKFVRDEDDRPKVAYNEFSDDIPVISLSGIDSPDDRDHIRRQVTEACEEYGIFQVVDHGIDSDIISTMARQSSQFFNLPAPEKQRFAAAEGKPGSFFVSSPFKGELVQNWRETVTQCTFPIKSGDYTLWPDKPEGWRSVTKEYSEKMMDLSHKLLGVLSEAMGLETEALSNACVTMDQRVMINYYPKCPQPDLTLGLPRHTDPGTITLLYQDLVGGLQATRDDGKTWITVPPIPGALVVNLGDHAFYASNGRFTSAEHRAVVNSNQSRLSIATFQYPTAEAMVYPLAIREGETAVMEEAITFAEMYRRKMSSDIERPKHKKVDGKMDKSKLESRPMEEIFV

SEQ ID NO: 9 - DNA, 1083 bp, Dianthus hybrida
  source 1..1083: mol_type = genomic DNA
atgacaaaggaaacaccctcgaccgtaacggtatgggaaaacgagacatccgtcaagcaaaagtttgtacgagatgaggacgaccgccctaaggtcgcctacaacgaattcagcgatgaaattcctgtcatttcgttgaatggtattgacaccgacaatgagagggcccacattcgtagcaagatcaccgaggcttgcgagacgtggggcatctttcaagtcgtggaccatggggttgaccctaatctcgtatctgaaatggctcgactttctaccgagtttttcaatttgccgattcacgagaagctccgctttggtgcttctgacggtaagcctggcagcttctttgtgtcgagcccctttaagggggagctagtgaaaaactggagggagacggtgacacaatgcacgtacccaatcaagagcggagactacaccctatggccggattcaccggacggttggaaaaatgtgacaaaagagtacagtgaaaaaatgatggacctaacacacaagctccttggggttttgtccgaggctatgggtctggaaaccgaagccttaagcaaggcgtgtgtcgatatggaccaaagggttatgatcaattactaccctaagtgcccgcaacctgacctcacccttggtctaccccgccacactgatcctggtaccatcacgcttttgtaccaggaccaggttggcggtctccaagctactcgcgatgatggcaagtcttggattactgtcccgcctgttgctggtgcccttgtcgtcaaccttggtgatcacgcctactatgtgagcaacgggaggttcacgagtgctgaacacagagcagtggtgaactcaaaccagagcaggctatcgatagcgacattccagtatccgacagccgaggcaaccatctacccattagcgattcgagaaggcgaggaacctgtgatggaagaagccatcacttttgcggaaatgtataggagaaagatgagctcggatatcgagcgtcctaagcttaagaagttggatggtacaatggacaagtccaagttagaagctagagctattggagaaatcttcgtgtag

SEQ ID NO: 10 - protein, 360 aa, Dianthus hybrida
MTKETPSTVTVWENETSVKQKFVRDEDDRPKVAYNEFSDEIPVISLNGIDTDNERAHIRSKITEACETWGIFQVVDHGVDPNLVSEMARLSTEFFNLPIHEKLRFGASDGKPGSFFVSSPFKGELVKNWRETVTQCTYPIKSGDYTLWPDSPDGWKNVTKEYSEKMMDLTHKLLGVLSEAMGLETEALSKACVDMDQRVMINYYPKCPQPDLTLGLPRHTDPGTITLLYQDQVGGLQATRDDGKSWITVPPVAGALVVNLGDHAYYVSNGRFTSAEHRAVVNSNQSRLSIATFQYPTAEATIYPLAIREGEEPVMEEAITFAEMYRRKMSSDIERPKLKKLDGTMDKSKLEARAIGEIFV

SEQ ID NO: 11 - DNA, 1080 bp, Dianthus caryophyllus L.
  source 1..1080: mol_type = genomic DNA
atgacaaaggaagcaccctcgaccgtaacggtatgggaaaacgagacatccgtcaagcaaaagtttgtacgagatgaggacgaccgccctaaggtcgcctacaacgaattcagcgatgaaattcctgtcatttcgttgaatggtattgacacagacaatgagagagcccacattcgtagcaagatcaccgaggcttgcgagacgtggggcatctttcaagtcgtggaccatgggtttgatcctaatctcgtatctgaaatggctcgactttctaccgagtttttcaatttgccgattcacgagaagctccgctttggtgcttctgacggtaagcctggcagcttctttgtgtcgagcccctttaagggggagctagtgaaaaactggagggagacggtgacacaatgcacgtacccaatcaagagcggagactacaccctatggccggattcaccggacggttggaaaaatgtgacaaaagagtacagtgaaaaaatgatggacctaacacacaagctccttggggttttgtccgaggctatgggtctggaaactgaagccttaagcaaggcgtgtgtcgatatggaccaaagggttatgatcaattactaccctaagtgcccgcaacctgacctcacccttggtctaccccgccacactgatcctggtaccatcacgcttttgtaccaggaccaggttggcggtctccaagctactcgcgatgatggcaagtcttggattactgtcccgcctgttgctggtgcccttgtcgtcaaccttggtgatcacgcctactatgtgagcaacgggaggttcacgagtgctgaacacagagcagtggtgaactcaaaccagagcaggctatctatagcgacattccagtatccgacagccgaggcaaccatctacccattagcgattcgagaaggcgaggaacctgtgatggaagaagccatcacttttgcggaaatgtataggagaaagatgagctcggatatcgagcgtcctaagcagaagttggatggtacaatggacaagtccaagttagaagctagagctattggagaaatcttcgtgtaa

SEQ ID NO: 12 - protein, 359 aa, Dianthus caryophyllus L.
MTKEAPSTVTVWENETSVKQKFVRDEDDRPKVAYNEFSDEIPVISLNGIDTDNERAHIRSKITEACETWGIFQVVDHGFDPNLVSEMARLSTEFFNLPIHEKLRFGASDGKPGSFFVSSPFKGELVKNWRETVTQCTYPIKSGDYTLWPDSPDGWKNVTKEYSEKMMDLTHKLLGVLSEAMGLETEALSKACVDMDQRVMINYYPKCPQPDLTLGLPRHTDPGTITLLYQDQVGGLQATRDDGKSWITVPPVAGALVVNLGDHAYYVSNGRFTSAEHRAVVNSNQSRLSIATFQYPTAEATIYPLAIREGEEPVMEEAITFAEMYRRKMSSDIERPKQKLDGTMDKSKLEARAIGEIFV

SEQ ID NO: 13 - DNA, 25 bp, synthetic construct
  source 1..25: mol_type = other DNA
atgacaaaagaggaatcaataaccg

SEQ ID NO: 14 - DNA, 23 bp, synthetic construct
  source 1..23: mol_type = other DNA
tcaaacaaagatctcgccgatgg

SEQ ID NO: 15 - DNA, 24 bp, synthetic construct
  source 1..24: mol_type = other DNA
atgacaaaagaaaaggcaacaacg

SEQ ID NO: 16 - DNA, 24 bp, synthetic construct
  source 1..24: mol_type = other DNA
ttaaataaagatggcgtcaatggg

SEQ ID NO: 17 - DNA, 29 bp, synthetic construct
  source 1..29: mol_type = other DNA
atgacaaaagaagataaaaaaaatgttac

SEQ ID NO: 18 - DNA, 25 bp, synthetic construct
  source 1..25: mol_type = other DNA
ttagataaagatctcattaatggcc

SEQ ID NO: 19 - DNA, 25 bp, synthetic construct
  source 1..25: mol_type = other DNA
atgacaaaggaaacaccctcgaccg

SEQ ID NO: 20 - DNA, 24 bp, synthetic construct
  source 1..24: mol_type = other DNA
ctacacgaagatttctccaatagc

SEQ ID NO: 21 - DNA, 26 bp, synthetic construct
  source 1..26: mol_type = other DNA
atgcctcaagaagagtcaataataac

SEQ ID NO: 22 - DNA, 25 bp, synthetic construct
  source 1..25: mol_type = other DNA
tcaaacaaagatctcttccatgggc